European Patent Specification EP 3 802 864 B1, published September 30, 2026. Title: METHODS OF PRODUCING NUCLEIC ACID LIBRARIES AND COMPOSITIONS AND KITS FOR PRACTICING SAME. Applicant: The Regents of the University of California Green, Richard Kapp, Joshua. The sequence listing filed with the application follows.

SEQUENCE LISTING (4 sequences)

SEQ ID NO: 1 - DNA, 33 bp, Artificial Sequence
  Synthetic sequence
acactctttccctacacgacgctcttccgatct

SEQ ID NO: 2 - DNA, 40 bp, Artificial Sequence
  Synthetic sequence
  misc_feature (1)..(7): n is a, c, g, or t
nnnnnnnagatcggaagagcgtcgtgtagggaaagagtgt

SEQ ID NO: 3 - DNA, 34 bp, Artificial Sequence
  Synthetic sequence
agatcggaagagcacacgtctgaactccagtcac

SEQ ID NO: 4 - DNA, 41 bp, Artificial Sequence
  Synthetic sequence
  misc_feature (35)..(41): n is a, c, g, or t
gtgactggagttcagacgtgtgctcttccgatctnnnnnnn